European Patent Specification EP 2 459 585 B1, published September 4, 2024. Title: INFLUENZA VIRUSES AND USES THEREOF. Applicant: Mount Sinai School of Medicine of New York University Palese, Peter Garcia-Sastre, Adolfo Gao, Qinshan. The sequence listing filed with the application follows.

SEQUENCE LISTING (136 sequences)

SEQ ID NO: 1 - DNA, 27 bp, Influenza PR8 virus
  3 prime non-coding region (NCR) of PB2 Packaging Sequences of PR8
agcgaaagcaggtcaattatattcaat

SEQ ID NO: 2 - DNA, 125 bp, Influenza PR8 virus
  3 prime proximal coding region (NCR) of PB2 Packaging Sequences of PR8
ttggaaagaataaaagaactaagaaatctattgtcgcagtctcgcacccgcgagatactcacaaaaaccaccgtggaccatttggccataatcaagaagtacacatcaggaagacaggagaagaa

SEQ ID NO: 3 - DNA, 158 bp, Artificial Sequence
  PB2 Packaging Sequences of PR8 with NheI restriction enzyme recognition site
agcgaaagcaggtcaattatattcaatttggaaagaataaaagaactaagaaatctattgtcgcagtctcgcacccgcgagatactcacaaaaaccaccgtggaccatttggccataatcaagaagtacacatcaggaagacaggagaagaagctagc

SEQ ID NO: 4 - DNA, 34 bp, Influenza PR8 virus
  5 prime non-coding region (NCR) of PB2 Packaging Sequences of PR8
tgtcgaatagtttaaaaacgaccttgtttctact

SEQ ID NO: 5 - DNA, 130 bp, Influenza PR8 virus
  5 prime proximal coding region (NCR) of PB2 Packaging Sequences of PR8
gaaaggagagaaggctaatgtgctaattgggcaaggagacgtggtgttggtaatgaaacggaaacgggactctagcatacttactgacagccagacagcgaccaaaagaattcggatggccatcaattag

SEQ ID NO: 6 - DNA, 169 bp, Artificial Sequence
  PB2 Packaging Sequences of PR8 with XhoI restriction enzyme recognition site
ctcgagaaaggagagaaggctaatgtgctaattgggcaaggagacgtggtgttggtaatgaaacggaaacgggactctagcatacttactgacagccagacagcgaccaaaagaattcggatggccatcaattagtgtcgaatagtttaaaaacgaccttgtttctact

SEQ ID NO: 7 - DNA, 24 bp, Influenza PR8 virus
  3 prime non-coding region (NCR) of PB1 Packaging Sequences of PR8
agcgaaagcaggcaaaccatttga

SEQ ID NO: 8 - DNA, 123 bp, Influenza PR8 virus
  3 prime proximal coding region (NCR) of PB1 Packaging Sequences of PR8
ttggttgtcaatccgaccttacttttcttaaaagtgccagcacaaattgctataagcacaactttcccttatactggagaccctccttacagccttgggacaggaacaggatacaccttggtt

SEQ ID NO: 9 - DNA, 153 bp, Artificial Sequence
  PB1 Packaging Sequences of PR8 with NheI restriction enzyme recognition site
agcgaaagcaggcaaaccatttgattggttgtcaatccgaccttacttttcttaaaagtgccagcacaaattgctataagcacaactttcccttatactggagaccctccttacagccttgggacaggaacaggatacaccttggttgctagc

SEQ ID NO: 10 - DNA, 42 bp, Influenza PR8 virus
  5 prime non-coding region (NCR) of PB1 Packaging Sequences of PR8
tgaatttagcttgtccttcatgaaaaaatgccttgtttctac

SEQ ID NO: 11 - DNA, 110 bp, Influenza PR8 virus
  5 prime proximal coding region (NCR) of PB1 Packaging Sequences of PR8
cccgaattgatgcacggattgatttcgaatctggaaggataaagaaagaagagttcactgagatcatgaagatctgttccaccattgaagagctcagacggcaaaaatag

SEQ ID NO: 12 - DNA, 159 bp, Artificial Sequence
  PB1 Packaging Sequences of PR8 with XhoI restriction enzyme recognition site
ctcgagcccgaattgatgcacggattgatttcgaatctggaaggataaagaaagaagagttcactgagatcatgaagatctgttccaccattgaagagctcagacggcaaaaatagtgaatttagcttgtccttcatgaaaaaatgccttgtttctact

SEQ ID NO: 13 - DNA, 24 bp, Influenza PR8 virus
  3 prime non-coding region (NCR) of PA Packaging Sequences of PR8
agcgaaagcaggtactgatccaaa

SEQ ID NO: 14 - DNA, 115 bp, Influenza PR8 virus
  3 prime proximal coding region (NCR) of PA Packaging Sequences of PR8
ttggaagattttgtgcgacattgcttcaatccgttgattgtcgagcttgcggaaaaaacattgaaagagtttggggaggacctgaaaatcgaaacaaacaaatttgcagcaattt

SEQ ID NO: 15 - DNA, 145 bp, Artificial Sequence
  PA Packaging Sequences of PR8 with NheI restriction enzyme recognition site
agcgaaagcaggtactgatccaaattggaagattttgtgcgacattgcttcaatccgttgattgtcgagcttgcggaaaaaacattgaaagagtttggggaggacctgaaaatcgaaacaaacaaatttgcagcaatttgctagc

SEQ ID NO: 16 - DNA, 58 bp, Influenza PR8 virus
  5 prime non-coding region (NCR) of PA Packaging Sequences of PR8
ttgtggcagtgctactatttgctatccatactgtccaaaaaagtaccttgtttctact

SEQ ID NO: 17 - DNA, 120 bp, Influenza PR8 virus
  5 prime proximal coding region (NCR) of PA Packaging Sequences of PR8
cctgggacctttgatcttggggggctatatgaagcaattgaggagtgcctgattaatgatccctgggttttgcttaatgcttcttggttcaactccttccttacacatgcattgagttag

SEQ ID NO: 18 - DNA, 184 bp, Artificial Sequence
  PA Packaging Sequences of PR8 with XhoI restriction enzyme recognition site
ctcgagcctgggacctttgatcttggggggctatatgaagcaattgaggagtgcctgattaatgatccctgggttttgcttaatgcttcttggttcaactccttccttacacatgcattgagttagttgtggcagtgctactatttgctatccatactgtccaaaaaagtaccttgtttctact

SEQ ID NO: 19 - DNA, 32 bp, Influenza PR8 virus
  3 prime non-coding region (NCR) of HA Packaging Sequences of PR8
agcaaaagcaggggaaaataaaaacaaccaaa

SEQ ID NO: 20 - DNA, 67 bp, Influenza PR8 virus
  3 prime proximal coding region (NCR) of HA Packaging Sequences of PR8
ttgaaggcaaacctactggtcctgttaagtgcacttgcagctgcagttgcagacacaatttgtatag

SEQ ID NO: 21 - DNA, 105 bp, Artificial Sequence
  HA Packaging Sequences of PR8 with NheI restriction enzyme recognition site
agcaaaagcaggggaaaataaaaacaaccaaattgaaggcaaacctactggtcctgttaagtgcacttgcagctgcagttgcagacacaatttgtataggctagc

SEQ ID NO: 22 - DNA, 45 bp, Influenza PR8 virus
  5 prime non-coding region (NCR) of HA Packaging Sequences of PR8
gattagaatttcagaaatatgaggaaaaacacccttgtttctact

SEQ ID NO: 23 - DNA, 105 bp, Influenza PR8 virus
  5 prime proximal coding region (NCR) of HA Packaging Sequences of PR8
atctactcaactgtcgccagttcactggtgcttttggtctccctgggggcaatcagtttctggatgtgttctaatggatctttgcagtgcagaatatgcatctga

SEQ ID NO: 24 - DNA, 156 bp, Artificial Sequence
  HA Packaging Sequences of PR8 with XhoI restriction enzyme recognition site
ctcgagatctactcaactgtcgccagttcactggtgcttttggtctccctgggggcaatcagtttctggatgtgttctaatggatctttgcagtgcagaatatgcatctgagattagaatttcagaaatatgaggaaaaacacccttgtttctact

SEQ ID NO: 25 - DNA, 45 bp, Influenza PR8 virus
  3 prime non-coding region (NCR) of NP Packaging Sequences of PR8
agcaaaagcagggtagataatcactcactgagtgacatcaaaatc

SEQ ID NO: 26 - DNA, 126 bp, Influenza PR8 virus
  3 prime proximal coding region (NCR) of NP Packaging Sequences of PR8
ttggcgtcccaaggcaccaaacggtcttacgaacagttggagactgttggagaacgccagattgccactgaaatcagagcatccgtcggaaaattgattggtggaattggacgattctacatccaa

SEQ ID NO: 27 - DNA, 177 bp, Artificial Sequence
  NP Packaging Sequences of PR8 with NheI restriction enzyme recognition site
agcaaaagcagggtagataatcactcactgagtgacatcaaaatcttggcgtcccaaggcaccaaacggtcttacgaacagttggagactgttggagaacgccagattgccactgaaatcagagcatccgtcggaaaattgattggtggaattggacgattctacatccaagctagc

SEQ ID NO: 28 - DNA, 23 bp, Influenza PR8 virus
  5 prime non-coding region (NCR) of NP Packaging Sequences of PR8
agaaaaatacccttgtttctact

SEQ ID NO: 29 - DNA, 120 bp, Influenza PR8 virus
  5 prime proximal coding region (NCR) of NP Packaging Sequences of PR8
gggcggggagtcttcgagctctcggacgaaaaggcagcgagcccgatcgtgccttcctttgacatgagtaatgaaggatcttatttcttcggagacaatgcagaggagtacgacaattaa

SEQ ID NO: 30 - DNA, 149 bp, Artificial Sequence
  NP Packaging Sequences of PR8 with XhoI restriction enzyme recognition site
ctcgaggggcggggagtcttcgagctctcggacgaaaaggcagcgagcccgatcgtgccttcctttgacatgagtaatgaaggatcttatttcttcggagacaatgcagaggagtacgacaattaaagaaaaatacccttgtttctact

SEQ ID NO: 31 - DNA, 20 bp, Influenza PR8 virus
  3 prime non-coding region (NCR) of NA Packaging Sequences of PR8
agcgaaagcaggggtttaaa

SEQ ID NO: 32 - DNA, 111 bp, Influenza PR8 virus
  3 prime proximal coding region (NCR) of NA Packaging Sequences of PR8
ttgaatccaaatcagaaaataacaaccattggatcaatctgtctggtagtcggactaattagcctaatattgcaaatagggaatataatctcaatttggattagccattca

SEQ ID NO: 33 - DNA, 137 bp, Artificial Sequence
  NA Packaging Sequences of PR8 with NheI restriction enzyme recognition site
agcgaaagcaggggtttaaattgaatccaaatcagaaaataacaaccattggatcaatctgtctggtagtcggactaattagcctaatattgcaaatagggaatataatctcaatttggattagccattcagctagc

SEQ ID NO: 34 - DNA, 28 bp, Influenza PR8 virus
  5 prime non-coding region (NCR) of NA Packaging Sequences of PR8
tctgttcaaaaaactccttgtttctact

SEQ ID NO: 35 - DNA, 157 bp, Influenza PR8 virus
  5 prime proximal coding region (NCR) of NA Packaging Sequences of PR8
gaggccgtgcttctgggttgaattaatcaggggacgacctaaagaaaaaacaatctggactagtgcgagcagcatttctttttgtggcgtgaatagtgatactgtagattggtcttggccagacggtgctgagttgccattcagcattgacaagtag

SEQ ID NO: 36 - DNA, 191 bp, Artificial Sequence
  NA Packaging Sequences of PR8 with XhoI restriction enzyme recognition site
ctcgaggaggccgtgcttctgggttgaattaatcaggggacgacctaaagaaaaaacaatctggactagtgcgagcagcatttctttttgtggcgtgaatagtgatactgtagattggtcttggccagacggtgctgagttgccattcagcattgacaagtagtctgttcaaaaaactccttgtttctact

SEQ ID NO: 37 - DNA, 25 bp, Influenza PR8 virus
  3 prime non-coding region (NCR) of M Packaging Sequences of PR8
agcgaaagcaggtagatattgaaag

SEQ ID NO: 38 - DNA, 255 bp, Influenza PR8 virus
  3 prime proximal coding region (NCR) of M Packaging Sequences of PR8
ttgagtcttctaaccgaggtcgaaacctacgtactctctatcatcccgtcaggccccctcaaagccgagatcgcacagagacttgaagttgtctttgcagggaagaacactgatcttgaggttctcttggattggctaaagacaagaccaatcctgtcacctctgactaaggggattttaggatttgtgttcacgctcaccgtgcccagtgagcgaggactgcagcgtagacgctttgtccaaattgcccttatt

SEQ ID NO: 39 - DNA, 286 bp, Artificial Sequence
  M Packaging Sequences of PR8 with NheI restriction enzyme recognition site
agcgaaagcaggtagatattgaaagttgagtcttctaaccgaggtcgaaacctacgtactctctatcatcccgtcaggccccctcaaagccgagatcgcacagagacttgaagttgtctttgcagggaagaacactgatcttgaggttctcttggattggctaaagacaagaccaatcctgtcacctctgactaaggggattttaggatttgtgttcacgctcaccgtgcccagtgagcgaggactgcagcgtagacgctttgtccaaattgcccttattgctagc

SEQ ID NO: 40 - DNA, 20 bp, Influenza PR8 virus
  5 prime non-coding region (NCR) of M Packaging Sequences of PR8
aaaactaccttgtttctact

SEQ ID NO: 41 - DNA, 215 bp, Influenza PR8 virus
  5 prime proximal coding region (NCR) of M Packaging Sequences of PR8
ctattgccgcaaatatcattgggatcttgcacttgacattgtggattcttgatcgtctttttttcaaatgcatttaccgtcgctttaaatacggactgaaaggagggccttctacggaaggagtgccaaagtctatgagggaagaatatcgaaaggaacagcagagtgctgtggatgctgacgatggtcattttgtcagcatagagctggagtaa

SEQ ID NO: 42 - DNA, 241 bp, Artificial Sequence
  M Packaging Sequences of PR8 with XhoI restriction enzyme recognition site
ctcgagctattgccgcaaatatcattgggatcttgcacttgacattgtggattcttgatcgtctttttttcaaatgcatttaccgtcgctttaaatacggactgaaaggagggccttctacggaaggagtgccaaagtctatgagggaagaatatcgaaaggaacagcagagtgctgtggatgctgacgatggtcattttgtcagcatagagctggagtaaaaaactaccttgtttctact

SEQ ID NO: 43 - DNA, 26 bp, Influenza PR8 virus
  3 prime non-coding region (NCR) of NS Packaging Sequences of PR8
agcaaaagcagggtgacaaagacata

SEQ ID NO: 44 - DNA, 77 bp, Influenza PR8 virus
  3 prime proximal coding region (NCR) of NS Packaging Sequences of PR8
ttggatccaaacactgtgtcaagctttcagctagattgctttctttggcttgtccgcaaacgagttgcagaccaaga

SEQ ID NO: 45 - DNA, 109 bp, Artificial Sequence
  NS Packaging Sequences of PR8 with NheI restriction enzyme recognition site
agcaaaagcagggtgacaaagacatattggatccaaacactgtgtcaagctttcagctagattgctttctttggcttgtccgcaaacgagttgcagaccaagagctagc

SEQ ID NO: 46 - DNA, 26 bp, Influenza PR8 virus
  5 prime non-coding region (NCR) of NS Packaging Sequences of PR8
taataaaaaacacccttgtttctact

SEQ ID NO: 47 - DNA, 102 bp, Influenza PR8 virus
  5 prime proximal coding region (NCR) of NS Packaging Sequences of PR8
ataacagagaatagttttgagcaaataacatttatgcaagccttacatctattgcttgaagtggagcaagagataagaactttctcgtttcagcttatttaa

SEQ ID NO: 48 - DNA, 134 bp, Artificial Sequence
  NS Packaging Sequences of PR8 with XhoI restriction enzyme recognition site
ctcgagataacagagaatagttttgagcaaataacatttatgcaagccttacatctattgcttgaagtggagcaagagataagaactttctcgtttcagcttatttaataataaaaaacacccttgtttctact

SEQ ID NO: 49 - DNA, 33 bp, Influenza PR8 virus
  Wild-type ORF 3 prime termini sequence
atggaaagaataaaagaactaagaaatctaatg

SEQ ID NO: 50 - DNA, 33 bp, Artificial Sequence
  mutated ORF 3 prime termini sequence for PB2
atggagcggatcaaggagttgcggaacttgatg

SEQ ID NO: 51 - DNA, 87 bp, Influenza PR8 virus
  Wild-type ORF 5 prime termini sequence for PB2
gtgttggtaatgaaacggaaacgggactctagcatacttactgacagccagacagcgaccaaaagaattcggatggccatcaattag

SEQ ID NO: 52 - DNA, 87 bp, Artificial Sequence
  mutated ORF 5 prime termini sequence for PB2
gtactagtgatgaagagaaagagagatagctctatcttgacggattcacaaacggcaactaagaggatccgtatggctattaactag

SEQ ID NO: 53 - DNA, 66 bp, Influenza PR8 virus
  Wild-type ORF 3 prime termini sequence for PB1
atggatgtcaatccgaccttacttttcttaaaagtgccagcacaaaatgctataagcacaactttc

SEQ ID NO: 54 - DNA, 66 bp, Artificial Sequence
  mutated ORF 3 prime termini sequence for PB1
atggacgttaacccaactctgttatttctgaaggtaccggcgcagaacgccatcagtacgaccttt

SEQ ID NO: 55 - DNA, 42 bp, Influenza PR8 virus
  Wild-type ORF 5 prime termini sequence for PB1
aagatctgttccaccattgaagagctcagacggcaaaaatag

SEQ ID NO: 56 - DNA, 42 bp, Artificial Sequence
  mutated ORF 5 prime termini sequence for PB1
aaaatttgcagtacaatcgaggaacttcggagacagaagtag

SEQ ID NO: 57 - DNA, 66 bp, Influenza PR8 virus
  Wild-type ORF 3 prime termini sequence for PA
atggaagattttgtgcgacaatgcttcaatccgatgattgtcgagcttgcggaaaaaacaatgaaa

SEQ ID NO: 58 - DNA, 66 bp, Artificial Sequence
  mutated ORF 3 prime termini sequence for PA
atggaggacttcgtaaggcagtgttttaacccaatgatcgttgaactcgcagagaagacgatgaag

SEQ ID NO: 59 - DNA, 45 bp, Influenza PR8 virus
  Wild-type ORF 5 prime termini sequence for PA
aatgcttcttggttcaactccttccttacacatgcattgagttag

SEQ ID NO: 60 - DNA, 45 bp, Artificial Sequence
  mutated ORF 5 prime termini sequence for PA
aacgccagctggtttaattcttttttgacgcacgcgctatcatag

SEQ ID NO: 61 - DNA, 48 bp, Influenza PR8 virus
  Wild-type ORF 3 prime termini sequence for HA
atgaaggcaaacctactggtcctgttaagtgcacttgcagctgcagat

SEQ ID NO: 62 - DNA, 48 bp, Artificial Sequence
  mutated ORF 3 prime termini sequence for HA
atgaaagcgaatttgttagttttactgtccgcgttggcggccgcggac

SEQ ID NO: 63 - DNA, 90 bp, Influenza PR8 virus
  Wild-type ORF 5 prime termini sequence for HA
gccagttcactggtgcttttggtctccctgggggcaatcagtttctggatgtgttctaatggatctttgcagtgcagaatatgcatctga

SEQ ID NO: 64 - DNA, 90 bp, Artificial Sequence
  mutated ORF 5 prime termini sequence for HA
gcttccagcttagtattgctagttagtttaggagcgatttccttttggatgtgcagcaacgggagcctacaatgtcggatttgtatttga

SEQ ID NO: 65 - DNA, 60 bp, Influenza PR8 virus
  Wild-type ORF 3 prime termini sequence for NP
atggcgtcccaaggcaccaaacggtcttacgaacagatggagactgatggagaacgccag

SEQ ID NO: 66 - DNA, 60 bp, Artificial Sequence
  mutated ORF 3 prime termini sequence for NP
atggcaagtcagggtactaagagaagctatgagcaaatggaaaccgacggggagagacaa

SEQ ID NO: 67 - DNA, 63 bp, Influenza PR8 virus
  Wild-type ORF 5 prime termini sequence for NP
tttgacatgagtaatgaaggatcttatttcttcggagacaatgcagaggagtacgacaattaa

SEQ ID NO: 68 - DNA, 63 bp, Artificial Sequence
  mutated ORF 5 prime termini sequence for NP
ttcgatatgtccaacgaggggagctacttttttggggataacgcggaagaatatgataactaa

SEQ ID NO: 69 - DNA, 60 bp, Influenza PR8 virus
  Wild-type ORF 3 prime termini sequence for NA
atgaatccaaatcagaaaataacaaccattggatcaatctgtctggtagtcggactaatt

SEQ ID NO: 70 - DNA, 60 bp, Artificial Sequence
  mutated ORF 3 prime termini sequence for NA
atgaacccgaaccaaaagatcacgactatcgggagcatttgcttagtggttgggttgatc

SEQ ID NO: 71 - DNA, 60 bp, Influenza PR8 virus
  Wild-type ORF 5 prime termini sequence for NA
gatactgtagattggtcttggccagacggtgctgagttgccattcagcattgacaagtag

SEQ ID NO: 72 - DNA, 60 bp, Artificial Sequence
  mutated ORF 5 prime termini sequence for NA
gacaccgtagactggagctggccggatggcgccgaactaccgttttctatcgataaatag

SEQ ID NO: 73 - DNA, 63 bp, Influenza PR8 virus
  Wild-type ORF 3 prime termini sequence for M
atgagtcttctaaccgaggtcgaaacgtacgtactctctatcatcccgtcaggccccctcaaa

SEQ ID NO: 74 - DNA, 63 bp, Artificial Sequence
  mutated ORF 3 prime termini sequence for M
atgagcttgttgactgaagtcgaaacgtacgtattgagcattattccaagtggtcctttaaag

SEQ ID NO: 75 - DNA, 60 bp, Influenza PR8 virus
  Wild-type ORF 5 prime termini sequence for M
gaacagcagagtgctgtggatgctgacgatggtcattttgtcagcatagagctggagtaa

SEQ ID NO: 76 - DNA, 60 bp, Artificial Sequence
  mutated ORF 5 prime termini sequence for M
gagcaacaatccgccgtagacgccgatgacggccacttcgtttctatcgaattagaataa

SEQ ID NO: 77 - DNA, 36 bp, Influenza PR8 virus
  Wild-type ORF 3 prime termini sequence for NS
atggatccaaacactgtgtcaagctttcaggtagat

SEQ ID NO: 78 - DNA, 36 bp, Artificial Sequence
  mutated ORF 3 prime termini sequence for NS
atggacccgaataccgtaagttcttttcaggtagac

SEQ ID NO: 79 - DNA, 36 bp, Influenza PR8 virus
  Wild-type ORF 5 prime termini sequence for NS
caagagataagaactttctcgtttcagcttatttaa

SEQ ID NO: 80 - DNA, 36 bp, Artificial Sequence
  mutated ORF 5 prime termini sequence for NS
caggaaatccggacctttagcttccaattgatctaa

SEQ ID NO: 81 - DNA, 32 bp, Influenza virus A/WSN/33; identical to SEQ ID NO: 19
  3 prime NCR of Influenza virus A/WSN/33 NA gene segment

SEQ ID NO: 82 - DNA, 1698 bp, Influenza virus A/WSN/33
  ORF of Influenza virus A/WSN/33 NA gene segment
atgaaggcaaaactactggtcctgttatatgcatttgtagctacagatgcagacacaatatgtataggctaccatgcgaacaactcaaccgacactgttgacacaatattcgagaagaatgtggcagtgacacattctgttaacctgctcgaagacagacacaacgggaaactatgtaaattaaaaggaatagccccactacaattggggaaatgtaacatcaccggatggctcttgggaaatccagaatgcgactcactgcttccagcgagatcatggtcctacattgtagaaacaccaaactctgagaatggagcatgttatccaggagatttcatcgactatgaggaactgagggagcaattgagctcagtatcatcattagaaagattcgaaatatttcccaaggaaagttcatggcccaaccacacattcaacggagtaacagtatcatgctcccataggggaaaaagcagtttttacagaaatttgctatggctgacgaagaagggggattcatacccaaagctgaccaattcctatgtgaacaataaagggaaagaagtccttgtactatggggtgttcatcacccgtccagcagtgatgagcaacagagtctctatagtaatggaaatgcttatgtctctgtagcgtcttcaaattataacaggagattcaccccggaaatagctgcaaggcccaaagtaaaagatcaacatgggaggatgaactattactggaccttgctagaacccggagacacaataatatttgaggcaactggtaatctaatagcaccatggtatgctttcgcactgagtagagggtttgagtccggcatcatcacctcaaacgcgtcaatgcatgagtgtaacacgaagtgtcaaacaccccagggatctataaacagcaatctccctttccagaatatacacccagtcacaataggagagtgcccaaaatatgtcaggagtaccaaattgaggatggttacaggactaagaaacatcccatccattcaatacagaggtctatttggagccattgctggttttattgaggggggatggactggaatgatagatggatggtatggttatcatcatcagaatgaacagggatcaggctatgcagcggatcaaaaaagcacacagaatgccattaacgggattacaaacaaggtgaactctgttatcgagaaaatgaacactcaattcacagctgtgggtaaagaattcaacaacttagaaaaaaggatggaaaatttaaataaaaaagttgatgatgggtttctggacatttggacatataatgcagaattgttagttctactggaaaatgaaagaactttggatttccatgacttaaatgtgaagaatctgtacgagaaagtaaaaagccaattaaagaataatgccaaagaaatcggaaatgggtgttttgagttctaccacaagtgtgacaatgaatgcatggaaagtgtaagaaatgggacttatgattatccaaaatattcagaagaatcaaagttgaacagggaaaagatagatggagtgaaattggaatcaatgggggtgtatcagattctggcgatctactcaactgtcgccagttcactggtgcttttggtctccctgggggcaatcagtttctggatgtgttctaatgggtctttgcagtgcagaatatgcatctga

SEQ ID NO: 83 - DNA, 45 bp, Influenza virus A/WSN/33
  5 prime NCR of Influenza virus A/WSN/33 HA gene segment
gattaggatttcagaaatataaggaaaaacacccttgtttctact

SEQ ID NO: 84 - DNA, 1775 bp, Influenza virus A/WSN/33
  Influenza virus A/WSN/33 HA gene segment
agcaaaagcaggggaaaataaaaacaaccaaaatgaaggcaaaactactggtcctgttatatgcatttgtagctacagatgcagacacaatatgtataggctaccatgcgaacaactcaaccgacactgttgacacaatattcgagaagaatgtggcagtgacacattctgttaacctgctcgaagacagacacaacgggaaactatgtaaattaaaaggaatagccccactacaattggggaaatgtaacatcaccggatggctcttgggaaatccagaatgcgactcactgcttccagcgagatcatggtcctacattgtagaaacaccaaactctgagaatggagcatgttatccaggagatttcatcgactatgaggaactgagggagcaattgagctcagtatcatcattagaaagattcgaaatatttcccaaggaaagttcatggcccaaccacacattcaacggagtaacagtatcatgctcccataggggaaaaagcagtttttacagaaatttgctatggctgacgaagaagggggattcatacccaaagctgaccaattcctatgtgaacaataaagggaaagaagtccttgtactatggggtgttcatcacccgtccagcagtgatgagcaacagagtctctatagtaatggaaatgcttatgtctctgtagcgtcttcaaattataacaggagattcaccccggaaatagctgcaaggcccaaagtaaaagatcaacatgggaggatgaactattactggaccttgctagaacccggagacacaataatatttgaggcaactggtaatctaatagcaccatggtatgctttcgcactgagtagagggtttgagtccggcatcatcacctcaaacgcgtcaatgcatgagtgtaacacgaagtgtcaaacaccccagggatctataaacagcaatctccctttccagaatatacacccagtcacaataggagagtgcccaaaatatgtcaggagtaccaaattgaggatggttacaggactaagaaacatcccatccattcaatacagaggtctatttggagccattgctggttttattgaggggggatggactggaatgatagatggatggtatggttatcatcatcagaatgaacagggatcaggctatgcagcggatcaaaaaagcacacagaatgccattaacgggattacaaacaaggtgaactctgttatcgagaaaatgaacactcaattcacagctgtgggtaaagaattcaacaacttagaaaaaaggatggaaaatttaaataaaaaagttgatgatgggtttctggacatttggacatataatgcagaattgttagttctactggaaaatgaaagaactttggatttccatgacttaaatgtgaagaatctgtacgagaaagtaaaaagccaattaaagaataatgccaaagaaatcggaaatgggtgttttgagttctaccacaagtgtgacaatgaatgcatggaaagtgtaagaaatgggacttatgattatccaaaatattcagaagaatcaaagttgaacagggaaaagatagatggagtgaaattggaatcaatgggggtgtatcagattctggcgatctactcaactgtcgccagttcactggtgcttttggtctccctgggggcaatcagtttctggatgtgttctaatgggtctttgcagtgcagaatatgcatctgagattaggatttcagaaatataaggaaaaacacccttgtttctact

SEQ ID NO: 85 - DNA, 19 bp, Influenza virus A/WSN/33
  3 prime NCR of Influenza virus A/WSN/33 NA gene segment
agcgaaagcaggagtttaa

SEQ ID NO: 86 - DNA, 1362 bp, Influenza virus A/WSN/33
  ORF of Influenza virus A/WSN/33 NA gene segment
atgaatccaaaccagaaaataataaccattgggtcaatctgtatggtagtcggaataattagcctaatattgcaaataggaaatataatctcaatatggattagccattcaattcaaaccggaaatcaaaaccatactggaatatgcaaccaaggcagcattacctataaagttgttgctgggcaggactcaacttcagtgatattaaccggcaattcatctctttgtcccatccgtgggtgggctatacacagcaaagacaatggcataagaattggttccaaaggagacgtttttgtcataagagagccttttatttcatgttctcacttggaatgcaggaccttttttctgactcaaggcgccttactgaatgacaagcattcaagggggacctttaaggacagaagcccttatagggccttaatgagctgccctgtcggtgaagctccgtccccgtacaattcaaggtttgaatcggttgcttggtcagcaagtgcatgtcatgatggagtgggctggctaacaatcggaatttctggtccagatgatggagcagtggctgtattaaaatacaaccgcataataactgaaaccataaaaagttggaggaagaatatattgagaacacaagagtctgaatgtacctgtgtaaatggttcatgttttaccataatgaccgatggcccaagtgatgggctggcctcgtacaaaattttcaagatcgagaaggggaaggttactaaatcaatagagttgaatgcacctaattctcactacgaggaatgttcctgttaccctgataccggcaaagtgatgtgtgtgtgcagagacaattggcacggttcgaaccgaccatgggtgtccttcgaccaaaacctagattataaaataggatacatctgcagtggggttttcggtgacaacccgcgtcccaaagatggaacaggcagctgtggcccagtgtctgctgatggagcaaacggagtaaagggattttcatataagtatggcaatggtgtttggataggaaggactaaaagtgacagttccagacatgggtttgagatgatttgggatcctaatggatggacagagactgatagtaggttctctatgagacaagatgttgtggcaataactaatcggtcagggtacagcggaagtttcgttcaacatcctgagctaacagggctagactgtatgaggccttgcttctgggttgaattaatcagggggctacctgaggaggacgcaatctggactagtgggagcatcatttctttttgtggtgtgaatagtgatactgtagattggtcttggccagacggtgctgagttgccgttcaccattgacaagtag

SEQ ID NO: 87 - DNA, 28 bp, Influenza virus A/WSN/33
  5 prime NCR of Influenza virus A/WSN/33 NA gene segment
tttgttcaaaaaactccttgtttctact

SEQ ID NO: 88 - DNA, 1409 bp, Influenza virus A/WSN/33
  Influenza virus A/WSN/33 NA gene segment
agcgaaagcaggagtttaaatgaatccaaaccagaaaataataaccattgggtcaatctgtatggtagtcggaataattagcctaatattgcaaataggaaatataatctcaatatggattagccattcaattcaaaccggaaatcaaaaccatactggaatatgcaaccaaggcagcattacctataaagttgttgctgggcaggactcaacttcagtgatattaaccggcaattcatctctttgtcccatccgtgggtgggctatacacagcaaagacaatggcataagaattggttccaaaggagacgtttttgtcataagagagccttttatttcatgttctcacttggaatgcaggaccttttttctgactcaaggcgccttactgaatgacaagcattcaagggggacctttaaggacagaagcccttatagggccttaatgagctgccctgtcggtgaagctccgtccccgtacaattcaaggtttgaatcggttgcttggtcagcaagtgcatgtcatgatggagtgggctggctaacaatcggaatttctggtccagatgatggagcagtggctgtattaaaatacaaccgcataataactgaaaccataaaaagttggaggaagaatatattgagaacacaagagtctgaatgtacctgtgtaaatggttcatgttttaccataatgaccgatggcccaagtgatgggctggcctcgtacaaaattttcaagatcgagaaggggaaggttactaaatcaatagagttgaatgcacctaattctcactacgaggaatgttcctgttaccctgataccggcaaagtgatgtgtgtgtgcagagacaattggcacggttcgaaccgaccatgggtgtccttcgaccaaaacctagattataaaataggatacatctgcagtggggttttcggtgacaacccgcgtcccaaagatggaacaggcagctgtggcccagtgtctgctgatggagcaaacggagtaaagggattttcatataagtatggcaatggtgtttggataggaaggactaaaagtgacagttccagacatgggtttgagatgatttgggatcctaatggatggacagagactgatagtaggttctctatgagacaagatgttgtggcaataactaatcggtcagggtacagcggaagtttcgttcaacatcctgagctaacagggctagactgtatgaggccttgcttctgggttgaattaatcagggggctacctgaggaggacgcaatctggactagtgggagcatcatttctttttgtggtgtgaatagtgatactgtagattggtcttggccagacggtgctgagttgccgttcaccattgacaagtagtttgttcaaaaaactccttgtttctact

SEQ ID NO: 89 - DNA, 25 bp, Influenza virus A/WSN/33
  3 prime NCR of Influenza virus A/WSN/33 M gene segment
agcaaaagcaggtagatattgaaag

SEQ ID NO: 90 - DNA, 982 bp, Influenza virus A/WSN/33
  ORF of Influenza virus A/WSN/33 M gene segment
atgagtcttctaaccgaggtcgaaacgtacgttctctctatcgtcccgtcaggccccctcaaagccgagatcgcacagagacttgaagatgtctttgcagggaagaacaccgatcttgaggttctcatggaatggctaaagacaagaccaatcctgtcacctctgactaaggggattttaggatttgtgttcacgctcaccgtgcccagtgagcggggactgcagcgtagacgctttgtccaaaatgctcttaatgggaacggagatccaaataacatggacaaagcagttaaactgtataggaagcttaagagggagataacattccatggggccaaagaaatagcactcagttattctgctggtgcacttgccagttgtatgggcctcatatacaacaggatgggggctgtggccactgaagtggcatttggcctggtatgcgcaacctgtgaacagattgctgactcccagcatcggtctcataggcaaatggtgacaacaaccaatccactaatcagacatgagaacagaatggttctagccagcactacagctaaggctatggagcaaatggctggatcgagtgagcaagcagcagaggccatggatattgctagtcaggccaggcaaatggtgcaggcgatgagaaccattgggactcatcctagctccagtactggtctaaaagatgatcttcttgaaaatttgcaggcctatcagaaacgaatgggggtgcagatgcaacgattcaagtgatcctctcgttattgcagcaaatatcattgggatcttgcacttgatattgtggattcttgatcgtctttttttcaaatgcatttatcgtcgctttaaatacggtttgaaaagagggccttctacggaaggagtgccagagtctatgagggaagaatatcgaaaggaacagcagaatgctgtggatgttgacgatggtcattttgtcaacatagagctggagtaa

SEQ ID NO: 91 - DNA, 20 bp, Influenza virus A/WSN/33
  5 prime NCR of Influenza virus A/WSN/33 M gene segment
aaaactaccttgtttctact

SEQ ID NO: 92 - DNA, 1027 bp, Influenza virus A/WSN/33
  Influenza virus A/WSN/33 M gene segment
agcaaaagcaggtagatattgaaagatgagtcttctaaccgaggtcgaaacgtacgttctctctatcgtcccgtcaggccccctcaaagccgagatcgcacagagacttgaagatgtctttgcagggaagaacaccgatcttgaggttctcatggaatggctaaagacaagaccaatcctgtcacctctgactaaggggattttaggatttgtgttcacgctcaccgtgcccagtgagcggggactgcagcgtagacgctttgtccaaaatgctcttaatgggaacggagatccaaataacatggacaaagcagttaaactgtataggaagcttaagagggagataacattccatggggccaaagaaatagcactcagttattctgctggtgcacttgccagttgtatgggcctcatatacaacaggatgggggctgtggccactgaagtggcatttggcctggtatgcgcaacctgtgaacagattgctgactcccagcatcggtctcataggcaaatggtgacaacaaccaatccactaatcagacatgagaacagaatggttctagccagcactacagctaaggctatggagcaaatggctggatcgagtgagcaagcagcagaggccatggatattgctagtcaggccaggcaaatggtgcaggcgatgagaaccattgggactcatcctagctccagtactggtctaaaagatgatcttcttgaaaatttgcaggcctatcagaaacgaatgggggtgcagatgcaacgattcaagtgatcctctcgttattgcagcaaatatcattgggatcttgcacttgatattgtggattcttgatcgtctttttttcaaatgcatttatcgtcgctttaaatacggtttgaaaagagggccttctacggaaggagtgccagagtctatgagggaagaatatcgaaaggaacagcagaatgctgtggatgttgacgatggtcattttgtcaacatagagctggagtaaaaaactaccttgtttctact

SEQ ID NO: 93 - DNA, 26 bp, Influenza virus A/WSN/33
  3 prime NCR of Influenza virus A/WSN/33 NS gene segment
agcaaaagcagggtgacaaagacata

SEQ ID NO: 94 - DNA, 838 bp, Influenza virus A/WSN/33
  ORF of Influenza virus A/WSN/33 NS gene segment
atggatccaaacactgtgtcaagctttcaggtagattgctttctttggcatgtccgcaaaagagttgcagaccaagaactaggtgattccccattccttgatcggcttcgccgagatcagaagtccctaagaggaagaggcagcactctcggtctggacatcgaaacagccacccgtgctggaaagcaaatagtggagcggattctgaaggaagaatccgatgaggcacttaaaatgaccatggcctctgtacctgcatcgcgctacctaactgacatgactcttgaggaaatgtcaaggcactggttcatgctcatgcccaagcagaaagtggcaggccctctttgtatcagaatggaccaggcgatcatggataagaacatcatactgaaagcgaacttcagtgtgatttttgaccggctggagactctaatattactaagggccttcaccgaagagggaacaattgttggcgaaatttcaccactgccttctcttccaggacatactgatgaggatgtcaaaaatgcagttggggtcctcatcggaggacttgaatggaataataacacagttcgagtctctgaaactctacagagattcgcttggagaagcagtaatgagaatgggagacctccactcactccaaaacagaaacgaaaaatggcgggaacaattaggtcagaagtttgaagaaataagatggttgattgaagaagtgagacacagactgaagataacagagaatagttttgagcaaataacatttatgcaagccttacaactattgcttgaagtggagcaagagataagaactttctcgtttcagcttatttaa

SEQ ID NO: 95 - DNA, 26 bp, Influenza virus A/WSN/33
  5 prime NCR of Influenza virus A/WSN/33 NS gene segment
taataaaaaacacccttgtttctact

SEQ ID NO: 96 - DNA, 890 bp, Influenza virus A/WSN/33
  Influenza virus A/WSN/33 NS gene segment
agcaaaagcagggtgacaaagacataatggatccaaacactgtgtcaagctttcaggtagattgctttctttggcatgtccgcaaaagagttgcagaccaagaactaggtgattccccattccttgatcggcttcgccgagatcagaagtccctaagaggaagaggcagcactctcggtctggacatcgaaacagccacccgtgctggaaagcaaatagtggagcggattctgaaggaagaatccgatgaggcacttaaaatgaccatggcctctgtacctgcatcgcgctacctaactgacatgactcttgaggaaatgtcaaggcactggttcatgctcatgcccaagcagaaagtggcaggccctctttgtatcagaatggaccaggcgatcatggataagaacatcatactgaaagcgaacttcagtgtgatttttgaccggctggagactctaatattactaagggccttcaccgaagagggaacaattgttggcgaaatttcaccactgccttctcttccaggacatactgatgaggatgtcaaaaatgcagttggggtcctcatcggaggacttgaatggaataataacacagttcgagtctctgaaactctacagagattcgcttggagaagcagtaatgagaatgggagacctccactcactccaaaacagaaacgaaaaatggcgggaacaattaggtcagaagtttgaagaaataagatggttgattgaagaagtgagacacagactgaagataacagagaatagttttgagcaaataacatttatgcaagccttacaactattgcttgaagtggagcaagagataagaactttctcgtttcagcttatttaataataaaaaacacccttgtttctact

SEQ ID NO: 97 - DNA, 24 bp, Influenza virus A/WSN/33
  3 prime NCR of Influenza virus A/WSN/33 PA gene segment
agcgaaagcaggtactgattcaaa

SEQ ID NO: 98 - DNA, 2151 bp, Influenza virus A/WSN/33
  ORF of Influenza virus A/WSN/33 PA gene segment
atggaagattttgtgcgacaatgcttcaatccgatgattgtcgagcttgcggaaaaggcaatgaaagagtatggagaggacctgaaaatcgaaacaaacaaatttgcagcaatatgcactcacttggaagtgtgcttcatgtattcagattttcacttcatcgatgagcaaggcgagtcaatagtcgtagaacttggcgatccaaatgcacttttgaagcacagatttgaaataatcgagggaagagatcgcacaatagcctggacagtaataaacagtatttgcaacactacaggggctgagaaaccaaagtttctaccagatttgtatgattacaagaagaatagattcatcgaaattggagtaacaaggagagaagttcacatatactatctggaaaaggccaataaaattaaatctgagaagacacacatccacattttctcattcactggggaggaaatggccacaaaggccgactacactctcgatgaagaaagcagggctaggatcaaaaccaggctattcaccataagacaagaaatggctagcagaggcctctgggattcctttcgtcagtccgagagaggcgaagagacaattgaagaaagatttgaaatcacaggaacaatgcgcaagcttgccgaccaaagtctcccgccaaacttctccagccttgaaaattttagagcctatgtggatggattcgaaccgaacggctacattgagggcaagctttctcaaatgtccaaagaagtaaatgctagaattgaaccttttttgaaatcaacaccacgaccacttagacttccggatgggcctccctgttctcagcggtccaaattcctgctgatggatgccttaaaattaagcattgaggacccaagtcatgagggagaggggataccgctatatgatgcaatcaaatgcatgagaacattctttggatggaaggaacccaatgttgttaaaccacacgaaaagggaataaatccaaattatcttctgtcatggaagcaagtactggcagaactgcaggacattgagaatgaggagaaaattccaaggactaaaaatatgaagaaaacgagtcagttaaagtgggcacttggtgagaacatggcaccagaaaaggtagactttgacgattgtaaagatgtaggcgatttgaagcaatatgatagtgatgaaccagaattgaggtcgcttgcaagttggattcagaatgagttcaacaaggcatgtgaactgaccgattcaagctggatagagctcgatgagattggagaagatgcggctccaattgaacacattgcaagcatgagaaggaattatttcacagcagaggtgtctcattgcagagccacagaatacataatgaagggggtgtacatcaatactgccttgcttaatgcatcctgtgcagcaatggatgatttccaattaattccaatgataagcaagtgtagaactaaggagggaaggcgaaagaccaatttgtacggtttcatcataaaaggaagatcccacttaaggaatgacaccgatgtggtaaactttgtgagcatggagttttccctcactgacccaagacttgaaccacacaaatgggagaagtactgtgttcttgaggtaggagatatgcttctaagaagtgccataggccatgtgtcaaggcctatgttcttgtatgtgaggacaaatggaacctcaaaaattaaaatgaaatgggggatggaaatgaggcgttgcctccttcagtcacttcaacaaatcgagagtatgattgaagctgagtcctctgtcaaggagaaagacatgaccaaagagttctttgaaaacaaatcagaaacatggcccgttggagagtcccccaaaggagtggaggaaggttccattgggaaggtctgcagaactttattggcaaagtcggtattcaacagcttgtatgcatctccacaactggaaggattttcagctgaatcaagaaaactgcttcttatcgttcaggctcttagggacaacctggaacctgggacctttgatcttggggggctatatgaagcaattgaggagtgcctgattaatgatccctgggttttgcttaatgcttcttggttcaactccttcctcacacatgcattgagatag

SEQ ID NO: 99 - DNA, 58 bp, Influenza virus A/WSN/33
  5 prime NCR of Influenza virus A/WSN/33 PA gene segment
ttgtggcaatgctactatttgctatccatactgtccaaaaaagtaccttgtttctact

SEQ ID NO: 100 - DNA, 2233 bp, Influenza virus A/WSN/33
  Influenza virus A/WSN/33 PA gene segment
agcgaaagcaggtactgattcaaaatggaagattttgtgcgacaatgcttcaatccgatgattgtcgagcttgcggaaaaggcaatgaaagagtatggagaggacctgaaaatcgaaacaaacaaatttgcagcaatatgcactcacttggaagtgtgcttcatgtattcagattttcacttcatcgatgagcaaggcgagtcaatagtcgtagaacttggcgatccaaatgcacttttgaagcacagatttgaaataatcgagggaagagatcgcacaatagcctggacagtaataaacagtatttgcaacactacaggggctgagaaaccaaagtttctaccagatttgtatgattacaagaagaatagattcatcgaaattggagtaacaaggagagaagttcacatatactatctggaaaaggccaataaaattaaatctgagaagacacacatccacattttctcattcactggggaggaaatggccacaaaggccgactacactctcgatgaagaaagcagggctaggatcaaaaccaggctattcaccataagacaagaaatggctagcagaggcctctgggattcctttcgtcagtccgagagaggcgaagagacaattgaagaaagatttgaaatcacaggaacaatgcgcaagcttgccgaccaaagtctcccgccaaacttctccagccttgaaaattttagagcctatgtggatggattcgaaccgaacggctacattgagggcaagctttctcaaatgtccaaagaagtaaatgctagaattgaaccttttttgaaatcaacaccacgaccacttagacttccggatgggcctccctgttctcagcggtccaaattcctgctgatggatgccttaaaattaagcattgaggacccaagtcatgagggagaggggataccgctatatgatgcaatcaaatgcatgagaacattctttggatggaaggaacccaatgttgttaaaccacacgaaaagggaataaatccaaattatcttctgtcatggaagcaagtactggcagaactgcaggacattgagaatgaggagaaaattccaaggactaaaaatatgaagaaaacgagtcagttaaagtgggcacttggtgagaacatggcaccagaaaaggtagactttgacgattgtaaagatgtaggcgatttgaagcaatatgatagtgatgaaccagaattgaggtcgcttgcaagttggattcagaatgagttcaacaaggcatgtgaactgaccgattcaagctggatagagctcgatgagattggagaagatgcggctccaattgaacacattgcaagcatgagaaggaattatttcacagcagaggtgtctcattgcagagccacagaatacataatgaagggggtgtacatcaatactgccttgcttaatgcatcctgtgcagcaatggatgatttccaattaattccaatgataagcaagtgtagaactaaggagggaaggcgaaagaccaatttgtacggtttcatcataaaaggaagatcccacttaaggaatgacaccgatgtggtaaactttgtgagcatggagttttccctcactgacccaagacttgaaccacacaaatgggagaagtactgtgttcttgaggtaggagatatgcttctaagaagtgccataggccatgtgtcaaggcctatgttcttgtatgtgaggacaaatggaacctcaaaaattaaaatgaaatgggggatggaaatgaggcgttgcctccttcagtcacttcaacaaatcgagagtatgattgaagctgagtcctctgtcaaggagaaagacatgaccaaagagttctttgaaaacaaatcagaaacatggcccgttggagagtcccccaaaggagtggaggaaggttccattgggaaggtctgcagaactttattggcaaagtcggtattcaacagcttgtatgcatctccacaactggaaggattttcagctgaatcaagaaaactgcttcttatcgttcaggctcttagggacaacctggaacctgggacctttgatcttggggggctatatgaagcaattgaggagtgcctgattaatgatccctgggttttgcttaatgcttcttggttcaactccttcctcacacatgcattgagatagttgtggcaatgctactatttgctatccatactgtccaaaaaagtaccttgtttctact

SEQ ID NO: 101 - DNA, 24 bp, Influenza virus A/WSN/33
  3 prime NCR of Influenza virus A/WSN/33 PB1 gene segment
agcgaaagcaggcaaaccatttga

SEQ ID NO: 102 - DNA, 2274 bp, Influenza virus A/WSN/33
  ORF of Influenza virus A/WSN/33 PB1 gene segment
atggatgtcaatccgactttacttttcttaaaagtgccagcacaaaatgctataagcacaactttcccttatactggagaccctccttacagccatgggacaggaacaggatacaccatggatactgtcaacaggacacatcagtactcagaaaggggaagatggacaacaaacaccgaaactggagcaccgcaactcaacccgattgatgggccactgccagaagacaatgaaccaagtggttatgcccaaacagattgtgtattggaagcaatggccttccttgaggaatcccatcctggtatctttgagacctcgtgtcttgaaacgatggaggttgttcagcaaacacgagtggacaagctgacacaaggccgacagacctatgactggactctaaataggaaccagcctgctgcaacagcattggccaacacaatagaagtgttcagatcaaatggcctcacggccaatgaatccggaaggctcatagacttccttaaggatgtaatggagtcaatgaacaaagaagaaatggagatcacaactcattttcagagaaagagacgagtgagagacaatatgactaagaaaatggtgacacagagaacaataggtaaaaggaagcagagattgaacaaaaggagttatctaattagggcattgaccctgaacacaatgaccaaagatgctgagagagggaagctaaaacggagagcaattgcaaccccagggatgcaaataagggggtttgtatactttgttgagacactagcaaggagtatatgtgagaaacttgaacaatcaggattgccagttggaggcaatgagaagaaagcaaagttggcaaatgttgtaaggaagatgatgaccaattctcaggacactgaaatttctttcaccatcactggagataacaccaaatggaacgaaaatcagaaccctcggatgtttttggccatgatcacatatataaccagaaatcagcccgaatggttcagaaatgttctaagtattgctccaataatgttctcaaacaaaatggcgagactgggaaaggggtacatgtttgagagcaagagtattaaaattagaactcaaatacctgcagaaatgctagcaagcatcgatttgaaatacttcaatgattcaactagaaagaagattgaaaaaatccggccgctcttaatagatgggactgcatcattgagccctggaatgatgatgggcatgttcaatatgttaagtactgtattaggcgtctccatcctgaatcttggacaaaagagacacaccaagactacttactggtgggatggtcttcaatcttctgatgattttgctctgattgtgaatgcacccaatcatgaagggattcaagccggagtcaacaggttttatcgaacctgtaagctacttggaattaatatgagcaagaaaaagtcttacataaacagaacaggtacatttgaattcacaagttttttctatcgttatgggtttgttgccaatttcagcatggagcttcccagctttggggtgtctgggatcaacgagtctgcggacatgagtattggagttactgtcatcaaaaacaatatgataaacaatgatcttggtccagcaaccgctcaaatggcccttcagctgttcatcaaagattacaggtacacgtaccggtgccatagaggtgacacacaaatacaaacccgaagatcatttgaaataaagaaactgtgggagcaaacccattccaaagctggactgctggtctccgacggaggcccaaatttatacaacattagaaatctccacattcctgaagtctgcttgaaatgggaattaatggatgaggattaccaggggcgtttatgcaacccactgaacccatttgtcaaccataaagacattgaatcagtgaacaatgcagtgataatgccagcacatggtccagccaaaaacatggagtatgatgctgttgcaacaacacactcctggatccccaaaagaaatcgatccatcttgaatacaagccaaagaggaatacttgaagatgaacaaatgtaccaaaagtgctgcaacttatttgaaaaattcttccccagcagttcatacagaagaccagtcgggatatccagtatggtggaggctatggtttccagagcccgaattgatgcacgaattgatttcgaatctggaaggataaagaaagaggagttcactgagatcatgaagatctgttccaccattgaagagctcagacggcaaaaatag

SEQ ID NO: 103 - DNA, 43 bp, Influenza virus A/WSN/33
  5 prime NCR of Influenza virus A/WSN/33 PB1 gene segment
tgaatttagcttgtccttcatgaaaaaatgccttgtttctact

SEQ ID NO: 104 - DNA, 2341 bp, Influenza virus A/WSN/33
  Influenza virus A/WSN/33 PB1 gene segment
agcgaaagcaggcaaaccatttgaatggatgtcaatccgactttacttttcttaaaagtgccagcacaaaatgctataagcacaactttcccttatactggagaccctccttacagccatgggacaggaacaggatacaccatggatactgtcaacaggacacatcagtactcagaaaggggaagatggacaacaaacaccgaaactggagcaccgcaactcaacccgattgatgggccactgccagaagacaatgaaccaagtggttatgcccaaacagattgtgtattggaagcaatggccttccttgaggaatcccatcctggtatctttgagacctcgtgtcttgaaacgatggaggttgttcagcaaacacgagtggacaagctgacacaaggccgacagacctatgactggactctaaataggaaccagcctgctgcaacagcattggccaacacaatagaagtgttcagatcaaatggcctcacggccaatgaatccggaaggctcatagacttccttaaggatgtaatggagtcaatgaacaaagaagaaatggagatcacaactcattttcagagaaagagacgagtgagagacaatatgactaagaaaatggtgacacagagaacaataggtaaaaggaagcagagattgaacaaaaggagttatctaattagggcattgaccctgaacacaatgaccaaagatgctgagagagggaagctaaaacggagagcaattgcaaccccagggatgcaaataagggggtttgtatactttgttgagacactagcaaggagtatatgtgagaaacttgaacaatcaggattgccagttggaggcaatgagaagaaagcaaagttggcaaatgttgtaaggaagatgatgaccaattctcaggacactgaaatttctttcaccatcactggagataacaccaaatggaacgaaaatcagaaccctcggatgtttttggccatgatcacatatataaccagaaatcagcccgaatggttcagaaatgttctaagtattgctccaataatgttctcaaacaaaatggcgagactgggaaaggggtacatgtttgagagcaagagtattaaaattagaactcaaatacctgcagaaatgctagcaagcatcgatttgaaatacttcaatgattcaactagaaagaagattgaaaaaatccggccgctcttaatagatgggactgcatcattgagccctggaatgatgatgggcatgttcaatatgttaagtactgtattaggcgtctccatcctgaatcttggacaaaagagacacaccaagactacttactggtgggatggtcttcaatcttctgatgattttgctctgattgtgaatgcacccaatcatgaagggattcaagccggagtcaacaggttttatcgaacctgtaagctacttggaattaatatgagcaagaaaaagtcttacataaacagaacaggtacatttgaattcacaagttttttctatcgttatgggtttgttgccaatttcagcatggagcttcccagctttggggtgtctgggatcaacgagtctgcggacatgagtattggagttactgtcatcaaaaacaatatgataaacaatgatcttggtccagcaaccgctcaaatggcccttcagctgttcatcaaagattacaggtacacgtaccggtgccatagaggtgacacacaaatacaaacccgaagatcatttgaaataaagaaactgtgggagcaaacccattccaaagctggactgctggtctccgacggaggcccaaatttatacaacattagaaatctccacattcctgaagtctgcttgaaatgggaattaatggatgaggattaccaggggcgtttatgcaacccactgaacccatttgtcaaccataaagacattgaatcagtgaacaatgcagtgataatgccagcacatggtccagccaaaaacatggagtatgatgctgttgcaacaacacactcctggatccccaaaagaaatcgatccatcttgaatacaagccaaagaggaatacttgaagatgaacaaatgtaccaaaagtgctgcaacttatttgaaaaattcttccccagcagttcatacagaagaccagtcgggatatccagtatggtggaggctatggtttccagagcccgaattgatgcacgaattgatttcgaatctggaaggataaagaaagaggagttcactgagatcatgaagatctgttccaccattgaagagctcagacggcaaaaatagtgaatttagcttgtccttcatgaaaaaatgccttgtttctact

SEQ ID NO: 105 - DNA, 27 bp, Influenza virus A/WSN/33
  3 prime NCR of Influenza virus A/WSN/33 PB2 gene segment
agcgaaagcaggtcaattatattcaat

SEQ ID NO: 106 - DNA, 2280 bp, Influenza virus A/WSN/33
  ORF of Influenza virus A/WSN/33 PB2 gene segment
atggaaagaataaaagaactaaggaatctaatgtcgcagtctcgcactcgcgagatactcacaaaaaccaccgtggaccatatggccataatcaagaagtacacatcaggaagacaggagaagaacccagcacttaggatgaaatggatgatggcaatgaaatatccaattacagcagacaagaggataacggaaatgattcctgagagaaatgagcagggacaaactttatggagtaaaatgaatgacgccggatcagaccgagtgatggtatcacctctggctgtgacatggtggaataggaatggaccagtgacaagtacagttcattatccaaaaatctacaaaacttattttgaaaaagtcgaaaggttaaaacatggaacctttggccctgtccattttagaaaccaagtcaaaatacgtcgaagagttgacataaatcctggtcatgcagatctcagtgccaaagaggcacaggatgtaatcatggaagttgttttccctaacgaagtgggagccaggatactaacatcggaatcgcaactaacgacaaccaaagagaagaaagaagaactccagggttgcaaaatttctcctctgatggtggcatacatgttggagagagaactggtccgcaaaacgagattcctcccagtggctggtggaacaagcagtgtgtacattgaagtgttgcatttgacccaaggaacatgctgggaacagatgtacactccaggaggggaggcgaggaatgatgatgttgatcaaagcttaattattgctgctagaaacatagtaagaagagccacagtgtcagcagatccactagcatctttattggagatgtgccacagcacgcagattggtggaataaggatggtaaacatccttaggcagaacccaacagaagagcaagccgtggatatttgcaaggctgcaatgggactgagaattagctcatccttcagttttggtggattcacatttaagagaacaagcggatcatcagtcaagagagaggaagaggtgcttacgggcaatcttcagacattgaagataagagtgcatgagggatatgaagagttcacaatggttgggagaagagcaacagctatactcagaaaagcaaccaggagattgattcagctgatagtgagtgggagggacgaacagtcgattgccgaagcaataattgtggccatggtattttcacaagaggattgtatgataaaagcagttagaggtgacctgaatttcgtcaatagggcgaatcagcgattgaaccccatgcaccaacttttgagacattttcagaaggatgcaaaggcgctctttcaaaattggggaattgaatccatcgacaatgtgatgggaatgatcgggatattgcccgacatgactccaagcaccgagatgtcaatgagaggagtgagaatcagcaaaatgggggtagatgagtattccagcgcggagaagatagtggtgagcattgaccgttttttgagagttagggaccaacgtgggaatgtactactgtctcccgaggaggtcagtgaaacacagggaacagagaaactgacaataacttactcatcgtcaatgatgtgggagattaatggtcctgaatcagtgttggtcaatacctatcagtggatcatcagaaactgggaaactgttaaaattcagtggtcccagaatcctacaatgctgtacaataaaatggaatttgagccatttcagtctttagttccaaaggccgttagaggccaatacagtgggtttgtgagaactctgttccaacaaatgagggatgtgcttgggacatttgataccgctcagataataaaacttcttcccttcgcagccgctccaccaaagcaaagtggaatgcagttctcctcattgactataaatgtgaggggatcaggaatgagaatacttgtaaggggcaattctccaatattcaactacaacaagaccactaaaagactcacagttctcggaaaggatgctggccctttaactgaagacccagatgaaggcacagctggagttgagtccgcagttctgagaggattcctcattctgggcaaagaagacaggagatatggaccagcattaagcataaatgaactgagcaaccttgcgaaaggagagaaggctaatgtgctaattgggcaaggagacgtggtgttggtaatgaaacggaaacggaactctagcatacttactgacagccagacagcgaccaaaagaattcggatggccatcaattag

SEQ ID NO: 107 - DNA, 34 bp, Influenza virus A/WSN/33; identical to SEQ ID NO: 4
  5 prime NCR of Influenza virus A/WSN/33 PB2 gene segment

SEQ ID NO: 108 - DNA, 2341 bp, Influenza virus A/WSN/33
  Influenza virus A/WSN/33 PB2 gene segment
agcgaaagcaggtcaattatattcaatatggaaagaataaaagaactaaggaatctaatgtcgcagtctcgcactcgcgagatactcacaaaaaccaccgtggaccatatggccataatcaagaagtacacatcaggaagacaggagaagaacccagcacttaggatgaaatggatgatggcaatgaaatatccaattacagcagacaagaggataacggaaatgattcctgagagaaatgagcagggacaaactttatggagtaaaatgaatgacgccggatcagaccgagtgatggtatcacctctggctgtgacatggtggaataggaatggaccagtgacaagtacagttcattatccaaaaatctacaaaacttattttgaaaaagtcgaaaggttaaaacatggaacctttggccctgtccattttagaaaccaagtcaaaatacgtcgaagagttgacataaatcctggtcatgcagatctcagtgccaaagaggcacaggatgtaatcatggaagttgttttccctaacgaagtgggagccaggatactaacatcggaatcgcaactaacgacaaccaaagagaagaaagaagaactccagggttgcaaaatttctcctctgatggtggcatacatgttggagagagaactggtccgcaaaacgagattcctcccagtggctggtggaacaagcagtgtgtacattgaagtgttgcatttgacccaaggaacatgctgggaacagatgtacactccaggaggggaggcgaggaatgatgatgttgatcaaagcttaattattgctgctagaaacatagtaagaagagccacagtgtcagcagatccactagcatctttattggagatgtgccacagcacgcagattggtggaataaggatggtaaacatccttaggcagaacccaacagaagagcaagccgtggatatttgcaaggctgcaatgggactgagaattagctcatccttcagttttggtggattcacatttaagagaacaagcggatcatcagtcaagagagaggaagaggtgcttacgggcaatcttcagacattgaagataagagtgcatgagggatatgaagagttcacaatggttgggagaagagcaacagctatactcagaaaagcaaccaggagattgattcagctgatagtgagtgggagggacgaacagtcgattgccgaagcaataattgtggccatggtattttcacaagaggattgtatgataaaagcagttagaggtgacctgaatttcgtcaatagggcgaatcagcgattgaaccccatgcaccaacttttgagacattttcagaaggatgcaaaggcgctctttcaaaattggggaattgaatccatcgacaatgtgatgggaatgatcgggatattgcccgacatgactccaagcaccgagatgtcaatgagaggagtgagaatcagcaaaatgggggtagatgagtattccagcgcggagaagatagtggtgagcattgaccgttttttgagagttagggaccaacgtgggaatgtactactgtctcccgaggaggtcagtgaaacacagggaacagagaaactgacaataacttactcatcgtcaatgatgtgggagattaatggtcctgaatcagtgttggtcaatacctatcagtggatcatcagaaactgggaaactgttaaaattcagtggtcccagaatcctacaatgctgtacaataaaatggaatttgagccatttcagtctttagttccaaaggccgttagaggccaatacagtgggtttgtgagaactctgttccaacaaatgagggatgtgcttgggacatttgataccgctcagataataaaacttcttcccttcgcagccgctccaccaaagcaaagtggaatgcagttctcctcattgactataaatgtgaggggatcaggaatgagaatacttgtaaggggcaattctccaatattcaactacaacaagaccactaaaagactcacagttctcggaaaggatgctggccctttaactgaagacccagatgaaggcacagctggagttgagtccgcagttctgagaggattcctcattctgggcaaagaagacaggagatatggaccagcattaagcataaatgaactgagcaaccttgcgaaaggagagaaggctaatgtgctaattgggcaaggagacgtggtgttggtaatgaaacggaaacggaactctagcatacttactgacagccagacagcgaccaaaagaattcggatggccatcaattagtgtcgaatagtttaaaaacgaccttgtttctact

SEQ ID NO: 109 - DNA, 45 bp, Influenza virus A/WSN/33
  3 prime NCR of Influenza virus A/WSN/33 NP gene segment
agcaaaagcagggtagataatcactcacagagtgacatcgaaatc

SEQ ID NO: 110 - DNA, 1497 bp, Influenza virus A/WSN/33
  ORF of Influenza virus A/WSN/33 NP gene segment
atggcgaccaaaggcaccaaacgatcttacgaacagatggagactgatggagaacgccagaatgccactgaaatcagagcatctgtcggaaaaatgattggtggaattggacgattctacatccaaatgtgcaccgaacttaaactcagtgattatgagggacggctgattcagaacagcttaacaatagagagaatggtgctctctgcttttgacgagaggaggaataaatatctagaagaacatcccagtgcggggaaagatcctaagaaaactggaggacctatatacaggagagtagatggaaagtggatgagagaactcatcctttatgacaaagaagaaataagacgaatctggcgccaagctaataatggtgacgatgcaacggctggtctgactcacatgatgatctggcactccaatttgaatgatgcaacttaccagaggacaagagctcttgttcgcacaggaatggatcccaggatgtgctcactgatgcagggttcaaccctccctaggaggtctggggccgcaggtgctgcagtcaaaggagttggaacaatggtgatggaattgatcagaatgatcaaacgtgggatcaatgatcggaacttctggaggggtgagaatggacggagaacaaggattgcttatgaaagaatgtgcaacattctcaaagggaaatttcaaacagctgcacaaagagcaatggtggatcaagtgagagagagccggaatccaggaaatgctgagttcgaagatctcatctttctagcacggtctgcactcatattgagagggtcagttgctcacaagtcctgcctgcctgcctgtgtgtatggacctgccgtagccagtggatacgactttgaaagagagggatactctctagtcggaatagaccctttcagactgcttcaaaacagccaagtatacagcctaatcagaccaaatgagaatccagcacacaagagtcaactggtgtggatggcatgccattctgctgcatttgaagatctaagagtatcaagcttcatcagagggacgaaagtggtcccaagagggaagctttccactagaggagttcaaattgcttccaatgaaaacatggagactatggaatcaagtacccttgaactgagaagcagatactgggccataaggaccagaagtggagggaacaccaatcaacagagggcttcctcgggccaaatcagcatacaacctacgttctcagtacagagaaatctcccttttgacagaccaaccattatggcagcattcactgggaatacagaggggagaacatctgacatgagaaccgaaatcataaggctgatggaaagtgcaagaccagaagatgtgtctttccaggggcggggagtcttcgagctctcggacgaaaaggcagcgagcccgatcgtgccctcctttgacatgagtaatgaaggatcttatttcttcggagacaatgcagaggagtacgacaattaa

SEQ ID NO: 111 - DNA, 23 bp, Influenza virus A/WSN/33
  5 prime NCR of Influenza virus A/WSN/33 NP gene segment
agaaaaatacccttgtttctact

SEQ ID NO: 112 - DNA, 1565 bp, Influenza virus A/WSN/33
  Influenza virus A/WSN/33 NP gene segment
agcaaaagcagggtagataatcactcacagagtgacatcgaaatcatggcgaccaaaggcaccaaacgatcttacgaacagatggagactgatggagaacgccagaatgccactgaaatcagagcatctgtcggaaaaatgattggtggaattggacgattctacatccaaatgtgcaccgaacttaaactcagtgattatgagggacggctgattcagaacagcttaacaatagagagaatggtgctctctgcttttgacgagaggaggaataaatatctagaagaacatcccagtgcggggaaagatcctaagaaaactggaggacctatatacaggagagtagatggaaagtggatgagagaactcatcctttatgacaaagaagaaataagacgaatctggcgccaagctaataatggtgacgatgcaacggctggtctgactcacatgatgatctggcactccaatttgaatgatgcaacttaccagaggacaagagctcttgttcgcacaggaatggatcccaggatgtgctcactgatgcagggttcaaccctccctaggaggtctggggccgcaggtgctgcagtcaaaggagttggaacaatggtgatggaattgatcagaatgatcaaacgtgggatcaatgatcggaacttctggaggggtgagaatggacggagaacaaggattgcttatgaaagaatgtgcaacattctcaaagggaaatttcaaacagctgcacaaagagcaatggtggatcaagtgagagagagccggaatccaggaaatgctgagttcgaagatctcatctttctagcacggtctgcactcatattgagagggtcagttgctcacaagtcctgcctgcctgcctgtgtgtatggacctgccgtagccagtggatacgactttgaaagagagggatactctctagtcggaatagaccctttcagactgcttcaaaacagccaagtatacagcctaatcagaccaaatgagaatccagcacacaagagtcaactggtgtggatggcatgccattctgctgcatttgaagatctaagagtatcaagcttcatcagagggacgaaagtggtcccaagagggaagctttccactagaggagttcaaattgcttccaatgaaaacatggagactatggaatcaagtacccttgaactgagaagcagatactgggccataaggaccagaagtggagggaacaccaatcaacagagggcttcctcgggccaaatcagcatacaacctacgttctcagtacagagaaatctcccttttgacagaccaaccattatggcagcattcactgggaatacagaggggagaacatctgacatgagaaccgaaatcataaggctgatggaaagtgcaagaccagaagatgtgtctttccaggggcggggagtcttcgagctctcggacgaaaaggcagcgagcccgatcgtgccctcctttgacatgagtaatgaaggatcttatttcttcggagacaatgcagaggagtacgacaattaaagaaaaatacccttgtttctact

SEQ ID NO: 113 - RNA, 131 nt, Artificial Sequence
  3 prime end 130 nt of the NS-HAmut-NS RNA
rucguuuucgucccacuguuucuguaugaccuagguuugugacacaguucgggagucgaucuaacgggagaaaccgaacaggcguuugcucaacgucugguucucggucguacuuucgcuuggacaaucaa

SEQ ID NO: 114 - DNA, 81 bp, Artificial Sequence
  forward primer used to amplify the HA ORF carried synonymous mutations
cagctagcatgaaagcgaatttgttagttttactgtccgcgttggcggccgcggacgcagacacaatatgtataggctacc

SEQ ID NO: 115 - DNA, 67 bp, Artificial Sequence
  reverse primer used to amplify the HA ORF carried synonymous mutations
ccaaaaggaaatcgctcctaaactaactagcaatactaagctggaagcgacagttgagtagatcgcc

SEQ ID NO: 116 - DNA, 73 bp, Artificial Sequence
  reverse primer used to amplify the HA ORF carried synonymous mutations
gtctcgagtcaaatacaaatccgacattgtaggctcccgttgctgcacatccaaaaggaaatcgctcctaaac

SEQ ID NO: 117 - DNA, 63 bp, Artificial Sequence
  forward primer used to introduced synonymous mutations into the NS ORF
cagctagcatggacccgaataccgtaagttcttttcaggtagactgctttctttggcatgtcc

SEQ ID NO: 118 - DNA, 57 bp, Artificial Sequence
  reverse primer used to introduced synonymous mutations into the NS ORF
gtctcgagttagatcaattggaagctaaaggtccggatttcctgctccacttcaagc

SEQ ID NO: 119 - DNA, 2668 bp, Artificial Sequence
  Chimeric influenza virus gene
agcgaaagcaggggtttaaattgaatccaaatcagaaaataacaaccattggatcaatctgtctggtagtcggactaattagcctaatattgcaaatagggaatataatctcaatttggattagccattcaattcaaactggaagtcaaaaccatactggaatttgcaaccaagctagcatggacgttaacccaactctgttatttctgaaggtaccggcgcagaacgccatcagtacgacctttccttatactggagaccctccttacagccatgggacaggaacaggatacaccatggatactgtcaacaggacacatcagtactcagaaaagggaagatggacaacaaacaccgaaactggagcaccgcaactcaacccgattgatgggccactgccagaagacaatgaaccaagtggttatgcccaaacagattgtgtattggaagcaatggctttccttgaggaatcccatcctggtatttttgaaaactcgtgtattgaaacgatggaggttgttcagcaaacacgagtagacaagctgacacaaggccgacagacctatgactggactctaaatagaaaccaacctgctgcaacagcattggccaacacaatagaagtgttcagatcaaatggcctcacggccaatgagtctggaaggctcatagacttccttaaggatgtaatggagtcaatgaaaaaagaagaaatggggatcacaactcattttcagagaaagagacgggtgagagacaatatgactaagaaaatgataacacagagaacaataggtaaaaagaagcagagattgaacaaaaggagttatctaattagagcattgaccctgaacacaatgaccaaagatgctgagagagggaagctaaaacggagagcaattgcaaccccagggatgcaaataagggggtttgtatactttgttgagacactggcaaggagtatatgtgagaaacttgaacaatcagggttgccagttggaggcaatgagaagaaagcaaagttggcaaatgttgtaaggaagatgatgaccaattctcaggacaccgaactttctttcaccatcactggagataacaccaaatggaacgaaaatcagaatcctcggatgtttttggccatgatcacatatatgacaagaaatcagcccgaatggttcagaaatgttctaagtattgctccaataatgttctcaaacaaaatggcgagactgggaaaagggtatatgtttgagagcaagagtatgaaacttagaactcaaatacctgcagaaatgctagcaagcatcgatttgaaatatttcaatgattcaacaagaaagaagattgaaaaaatccgaccgctcttaatagaggggactgcatcattgagccctggaatgatgatgggcatgttcaatatgttaagcactgtattaggcgtctccatcctgaatcttggacaaaagagatacaccaagactacttactggtgggatggtcttcaatcctctgacgattttgctctgattgtgaatgcacccaatcatgaagggattcaagccggagtcgacaggttttatcgaacctgtaagctacttggaatcaatatgagcaagaaaaagtcttacataaacagaacaggtacatttgaattcacaagttttttctatcgttatgggtttgttgccaatttcagcatggagctccccagttttggggtgtctgggatcaacgagtcagcggacatgagtattggagttactgtcatcaaaaacaatatgataaacaatgatcttggtccagcaacagctcaaatggcccttcagttgttcatcaaagattacaggtacacgtaccgatgccatagaggtgacacacaaatacaaacccgaagatcatttgaaataaagaaactgtgggagcaaacccgttccaaagctggactgctggtctccgacggaggcccaaatttatacaacattagaaatctccacattcctgaagtctgcctaaaatgggaattgatggatgaggattaccaggggcgtttatgcaacccactgaacccatttgtcagccataaagaaattgaatcaatgaacaatgcagtgatgatgccagcacatggtccagccaaaaacatggagtatgatgctgttgcaacaacacactcctggatccccaaaagaaatcgatccatcttgaatacaagtcaaagaggagtacttgaagatgaacaaatgtaccaaaggtgctgcaatttatttgaaaaattcttccccagcagttcatacagaagaccagtcgggatatccagtatggtggaggctatggtttccagagcccgaattgatgcacggattgatttcgaatctggaaggataaagaaagaagagttcactgagatcatgaaaatttgcagtacaatcgaggaacttcggagacagaagtagctcgagtgagctaacagggctagactgtatgaggccgtgcttctgggttgaattaatcaggggacgacctaaagaaaaaacaatctggactagtgcgagcagcatttctttttgtggcgtgaatagtgatactgtagattggtcttggccagacggtgctgagttgccattcagcattgacaagtagtctgttcaaaaaactccttgtttctact

SEQ ID NO: 120 - DNA, 2674 bp, Artificial Sequence
  Chimeric influenza virus gene
agcgaaagcaggggtttaaattgaatccaaatcagaaaataacaaccattggatcaatctgtctggtagtcggactaattagcctaatattgcaaatagggaatataatctcaatttggattagccattcaattcaaactggaagtcaaaaccatactggaatttgcaaccaagctagcatggagcggatcaaggagttgcggaacttgatgtcgcagtctcgcacccgcgagatactcacaaaaaccaccgtggaccatatggccataatcaagaagtacacatcaggaagacaggagaagaacccagcacttaggatgaaatggatgatggcaatgaaatatccaattacagcagacaagaggataacggaaatgattcctgagagaaatgagcaaggacaaactttatggagtaaaatgaatgatgcaggatcagaccgagtgatggtatcacctctggctgtgacatggtggaataggaatggaccaataacaaatacagttcattatccaaaaatctacaaaacttattttgaaagagtcgaaaggctaaagcatggaacctttggccctgtccattttagaaaccaagtcaaaatacgtcggagagttgacataaatcctggtcatgcagatctcagtgccaaggaggcacaggatgtaatcatggaagttgttttccctaacgaagtgggagccaggatactaacatcggaatcgcaactaacgataaccaaagagaagaaagaagaactccaggattgcaaaatttctcctttgatggttgcatacatgttggagagagaactggtccgcaaaacgagattcctcccagtggctggtggaacaagcagtgtgtacattgaagtgttgcatttgactcaaggaacatgctgggaacagatgtatactccaggaggggaagtgaggaatgatgatgttgatcaaagcttgattattgctgctaggaacatagtgagaagagctgcagtatcagcagatccactagcatctttattggagatgtgccacagcacacagattggtggaattaggatggtagacatccttaggcagaacccaacagaagagcaagccgtggatatatgcaaggctgcaatgggactgagaattagctcatccttcagttttggtggattcacatttaagagaacaagcggatcatcagtcaagagagaggaagaggtgcttacgggcaatcttcaaacattgaagataagagtgcatgagggatatgaagagttcacaatggttgggagaagagcaacagccatactcagaaaagcaaccaggagattgattcagctgatagtgagtgggagagacgaacagtcgattgccgaagcaataattgtggccatggtattttcacaagaggattgtatgataaaagcagtcagaggtgatctgaatttcgtcaatagggcgaatcagcgattgaatcctatgcatcaacttttaagacattttcagaaggatgcgaaagtgctttttcaaaattggggagttgaacctatcgacaatgtgatgggaatgattgggatattgccagacatgactccaagcatcgagatgtcaatgagaggagtgagaatcagcaaaatgggtgtagatgagtactccagcacggagagggtagtggtgagcattgaccgttttttgagaatccgggaccaacgaggaaatgtactactgtctcccgaggaggtcagtgaaacacagggaacagagaaactgacaataacttactcatcgtcaatgatgtgggagattaatggtcctgaatcagtgttggtcaatacctatcaatggatcatcagaaactgggaaactgttaaaattcagtggtcccagaaccctacaatgctatacaataaaatggaatttgaaccatttcagtctttagtacctaaggccattagaggccaatacagtgggtttgtaagaactctgttccaacaaatgagggatgtgcttgggacatttgataccgcacagataataaaacttcttcccttcgcagccgctccaccaaagcaaagtagaatgcagttctcctcatttactgtgaatgtgaggggatcaggaatgagaatacttgtaaggggcaattctcctgtattcaactataacaaggccacgaagagactcacagttctcggaaaggatgctggcactttaactgaagacccagatgaaggcacagctggagtggagtccgctgttctgaggggattcctcattctgggcaaagaagacaagagatatgggccagcactaagcatcaatgaactgagcaaccttgcgaaaggagagaaggctaatgtgctaattgggcaaggagacgtggtactagtgatgaagagaaagagagatagctctatcttgacggattcacaaacggcaactaagaggatccgtatggctattaactagctcgagtgagctaacagggctagactgtatgaggccgtgcttctgggttgaattaatcaggggacgacctaaagaaaaaacaatctggactagtgcgagcagcatttctttttgtggcgtgaatagtgatactgtagattggtcttggccagacggtgctgagttgccattcagcattgacaagtagtctgttcaaaaaactccttgtttctact

SEQ ID NO: 121 - DNA, 2545 bp, Artificial Sequence
  Chimeric influenza virus gene
agcgaaagcaggggtttaaattgaatccaaatcagaaaataacaaccattggatcaatctgtctggtagtcggactaattagcctaatattgcaaatagggaatataatctcaatttggattagccattcaattcaaactggaagtcaaaaccatactggaatttgcaaccaagctagcatggaggacttcgtaaggcagtgttttaacccaatgatcgttgaactcgcagagaagacgatgaaggagtatggggaggacctgaaaatcgaaacaaacaaatttgcagcaatatgcactcacttggaagtatgcttcatgtattcagattttcacttcatcaatgagcaaggcgagtcaataatcgtagaacttggtgatccaaatgcacttttgaagcacagatttgaaataatcgagggaagagatcgcacaatggcctggacagtagtaaacagtatttgcaacactacaggggctgagaaaccaaagtttctaccagatttgtatgattacaaggagaatagattcatcgaaattggagtaacaaggagagaagttcacatatactatctggaaaaggccaataaaattaaatctgagaaaacacacatccacattttctcgttcactggggaagaaatggccacaaaggcagactacactctcgatgaagaaagcagggctaggatcaaaaccagactattcaccataagacaagaaatggccagcagaggcctctgggattcctttcgtcagtccgagagaggagaagagacaattgaagaaaggtttgaaatcacaggaacaatgcgcaagcttgccgaccaaagtctcccgccgaacttctccagccttgaaaattttagagcctatgtggatggattcgaaccgaacggctacattgagggcaagctgtctcaaatgtccaaagaagtaaatgctagaattgaaccttttttgaaaacaacaccacgaccacttagacttccgaatgggcctccctgttctcagcggtccaaattcctgctgatggatgccttaaaattaagcattgaggacccaagtcatgaaggagagggaataccgctatatgatgcaatcaaatgcatgagaacattctttggatggaaggaacccaatgttgttaaaccacacgaaaagggaataaatccaaattatcttctgtcatggaagcaagtactggcagaactgcaggacattgagaatgaggagaaaattccaaagactaaaaatatgaagaaaacaagtcagctaaagtgggcacttggtgagaacatggcaccagaaaaggtagactttgacgactgtaaagatgtaggtgatttgaagcaatatgatagtgatgaaccagaattgaggtcgctagcaagttggattcagaatgagtttaacaaggcatgcgaactgacagattcaagctggatagagctcgatgagattggagaagatgtggctccaattgaacacattgcaagcatgagaaggaattatttcacatcagaggtgtctcactgcagagccacagaatacataatgaagggggtgtacatcaatactgccttgcttaatgcatcttgtgcagcaatggatgatttccaattaattccaatgataagcaagtgtagaactaaggagggaaggcgaaagaccaacttgtatggtttcatcataaaaggaagatcccacttaaggaatgacaccgacgtggtaaactttgtgagcatggagttttctctcactgacccaagacttgaaccacataaatgggagaagtactgtgttcttgagataggagatatgcttataagaagtgccataggccaggtttcaaggcccatgttcttgtatgtgagaacaaatggaacctcaaaaattaaaatgaaatggggaatggagatgaggcgttgcctcctccagtcacttcaacaaattgagagtatgattgaagctgagtcctctgtcaaagagaaagacatgaccaaagagttctttgagaacaaatcagaaacatggcccattggagagtcccccaaaggagtggaggaaagttccattgggaaggtctgcaggactttattagcaaagtcggtattcaacagcttgtatgcatctccacaactagaaggattttcagctgaatcaagaaaactgcttcttatcgttcaggctcttagggacaaccttgaacctgggacctttgatcttggggggctatatgaagcaattgaggagtgcctgattaatgatccctgggttttgcttaacgccagctggtttaattcttttttgacgcacgcgctatcatagctcgagtgagctaacagggctagactgtatgaggccgtgcttctgggttgaattaatcaggggacgacctaaagaaaaaacaatctggactagtgcgagcagcatttctttttgtggcgtgaatagtgatactgtagattggtcttggccagacggtgctgagttgccattcagcattgacaagtagtctgttcaaaaaactccttgtttctact

SEQ ID NO: 122 - DNA, 1032 bp, Artificial Sequence
  Chimeric influenza virus gene
agcgaaagcaggcaaaccatttgattggttgtcaatccgaccttacttttcttaaaagtgccagcacaaattgctataagcacaactttcccttatactggagaccctccttacagccttgggacaggaacaggatacaccttggttgctagcatggtgagcaagggcgaggagctgttcaccggggtggtgcccatcctggtcgagctggacggcgacgtaaacggccacaagttcagcgtgtccggcgagggcgagggcgatgccacctacggcaagctgaccctgaagttcatctgcaccaccggcaagctgcccgtgccctggcccaccctcgtgaccaccctgacctacggcgtgcagtgcttcagccgctaccccgaccacatgaagcagcacgacttcttcaagtccgccatgcccgaaggctacgtccaggagcgcaccatcttcttcaaggacgacggcaactacaagacccgcgccgaggtgaagttcgagggcgacaccctggtgaaccgcatcgagctgaagggcatcgacttcaaggaggacggcaacatcctggggcacaagctggagtacaactacaacagccacaacgtctatatcatggccgacaagcagaagaacggcatcaaggtgaacttcaagatccgccacaacatcgaggacggcagcgtgcagctcgccgaccactaccagcagaacacccccatcggcgacggccccgtgctgctgcccgacaaccactacctgagcacccagtccgccctgagcaaagaccccaacgagaagcgcgatcacatggtcctgctggagttcgtgaccgccgccgggatcactctcggcatggacgagctgtacaagtaactcgagcccgaattgatgcacggattgatttcgaatctggaaggataaagaaagaagagttcactgagatcatgaagatctgttccaccattgaagagctcagacggcaaaaatagtgaatttagcttgtccttcatgaaaaaatgccttgtttctact

SEQ ID NO: 123 - DNA, 1047 bp, Artificial Sequence
  Chimeric influenza virus gene
agcgaaagcaggtcaattatattcaatttggaaagaataaaagaactaagaaatctattgtcgcagtctcgcacccgcgagatactcacaaaaaccaccgtggaccatttggccataatcaagaagtacacatcaggaagacaggagaagaagctagcatggtgagcaagggcgaggagctgttcaccggggtggtgcccatcctggtcgagctggacggcgacgtaaacggccacaagttcagcgtgtccggcgagggcgagggcgatgccacctacggcaagctgaccctgaagttcatctgcaccaccggcaagctgcccgtgccctggcccaccctcgtgaccaccctgacctacggcgtgcagtgcttcagccgctaccccgaccacatgaagcagcacgacttcttcaagtccgccatgcccgaaggctacgtccaggagcgcaccatcttcttcaaggacgacggcaactacaagacccgcgccgaggtgaagttcgagggcgacaccctggtgaaccgcatcgagctgaagggcatcgacttcaaggaggacggcaacatcctggggcacaagctggagtacaactacaacagccacaacgtctatatcatggccgacaagcagaagaacggcatcaaggtgaacttcaagatccgccacaacatcgaggacggcagcgtgcagctcgccgaccactaccagcagaacacccccatcggcgacggccccgtgctgctgcccgacaaccactacctgagcacccagtccgccctgagcaaagaccccaacgagaagcgcgatcacatggtcctgctggagttcgtgaccgccgccgggatcactctcggcatggacgagctgtacaagtaactcgagaaaggagagaaggctaatgtgctaattgggcaaggagacgtggtgttggtaatgaaacggaaacgggactctagcatacttactgacagccagacagcgaccaaaagaattcggatggccatcaattagtgtcgaatagtttaaaaacgaccttgtttctact

SEQ ID NO: 124 - DNA, 1049 bp, Artificial Sequence
  Chimeric influenza virus gene
agcgaaagcaggtactgatccaaattggaagattttgtgcgacattgcttcaatccgttgattgtcgagcttgcggaaaaaacattgaaagagtttggggaggacctgaaaatcgaaacaaacaaatttgcagcaatttgctagcatggtgagcaagggcgaggagctgttcaccggggtggtgcccatcctggtcgagctggacggcgacgtaaacggccacaagttcagcgtgtccggcgagggcgagggcgatgccacctacggcaagctgaccctgaagttcatctgcaccaccggcaagctgcccgtgccctggcccaccctcgtgaccaccctgacctacggcgtgcagtgcttcagccgctaccccgaccacatgaagcagcacgacttcttcaagtccgccatgcccgaaggctacgtccaggagcgcaccatcttcttcaaggacgacggcaactacaagacccgcgccgaggtgaagttcgagggcgacaccctggtgaaccgcatcgagctgaagggcatcgacttcaaggaggacggcaacatcctggggcacaagctggagtacaactacaacagccacaacgtctatatcatggccgacaagcagaagaacggcatcaaggtgaacttcaagatccgccacaacatcgaggacggcagcgtgcagctcgccgaccactaccagcagaacacccccatcggcgacggccccgtgctgctgcccgacaaccactacctgagcacccagtccgccctgagcaaagaccccaacgagaagcgcgatcacatggtcctgctggagttcgtgaccgccgccgggatcactctcggcatggacgagctgtacaagtaactcgagcctgggacctttgatcttggggggctatatgaagcaattgaggagtgcctgattaatgatccctgggttttgcttaatgcttcttggttcaactccttccttacacatgcattgagttagttgtggcagtgctactatttgctatccatactgtccaaaaaagtaccttgtttctact

SEQ ID NO: 125 - DNA, 2013 bp, Artificial Sequence
  Chimeric influenza virus gene
agcgaaagcaggcaaaccatttgattggttgtcaatccgaccttacttttcttaaaagtgccagcacaaattgctataagcacaactttcccttatactggagaccctccttacagccttgggacaggaacaggatacaccttggttgctagcatgaagaccatcattgctttgagctacattttctgtctggctctcggccaagaccttccaggaaatgacaacagcacagcaacgctgtgcctgggacatcatgcggtgccaaacggaacactagtgaaaacaatcacagatgatcagattgaagtgactaatgctactgagctagttcagagctcctcaacggggaaaatatgcaacaatcctcatcgaatccttgatggaatagactgcacactgatagatgctctattgggggaccctcattgtgatgtttttcaaaatgagacatgggaccttttcgttgaacgcagcaaagctttcagcaactgttacccttatgatgtgccagattatgcctcccttaggtcactagttgcctcgtcaggcactctggagtttatcactgagggtttcacttggactggggtcactcagaatgggggaagcaatgcttgcaaaaggggacctggtagcggttttttcagtagactgaactggttgaccaaatcaggaagcacatatccagtgctgaacgtgactatgccaaacaatgacaattttgacaaactatacatttggggggttcaccacccgagcacgaaccaagaacaaaccagcctgtatgttcaagcatcagggagagtcacagtctctaccaggagaagccagcaaactataatcccgaatatcgggtccagaccctgggtaaggggtctgtctagtagaataagcatctattggacaatagttaagccgggagacgtactggtaattaatagtaatgggaacctaatcgctcctcggggttatttcaaaatgcgcactgggaaaagctcaataatgaggtcagatgcacctattgatacctgtatttctgaatgcatcactccaaatggaagcattcccaatgacaagccctttcaaaacgtaaacaagatcacatatggagcatgccccaagtatgttaagcaaaacaccctgaagttggcaacagggatgcggaatgtaccagagaaacaaactagaggcctattcggcgcaatagcaggtttcatagaaaatggttgggagggaatgatagacggttggtacggtttcaggcatcaaaattctgagggcacaggacaagcagcagatcttaaaagcactcaagcagccatcgaccaaatcaatgggaaattgaacagggtaatcgagaagacgaacgagaaattccatcaaatcgaaaaggaattctcagaagtagaagggagaattcaggacctcgagaaatacgttgaagacactaaaatagatctctggtcttacaatgcggagcttcttgtcgctctggagaatcaacatacaattgacctgactgactcggaaatgaacaagctgtttgaaaaaacagggaggcaactgagggaaaatgctgaagacatgggcaatggttgcttcaaaatataccacaaatgtgacaacgcttgcatagagtcaatcagaaatgggacttatgaccatgatgtatacagagacgaagcattaaacaaccggtttcagatcaaaggtgttgaactgaagtctggatacaaagactggatcctgtggatttcctttgccatatcatgctttttgctttgtgttgttttgctggggttcatcatgtgggcctgccagagaggcaacattaggtgcaacatttgcatttgactcgagcccgaattgatgcacggattgatttcgaatctggaaggataaagaaagaagagttcactgagatcatgaagatctgttccaccattgaagagctcagacggcaaaaatagtgaatttagcttgtccttcatgaaaaaatgccttgtttctact

SEQ ID NO: 126 - DNA, 2028 bp, Artificial Sequence
  Chimeric influenza virus gene
agcgaaagcaggtcaattatattcaatttggaaagaataaaagaactaagaaatctattgtcgcagtctcgcacccgcgagatactcacaaaaaccaccgtggaccatttggccataatcaagaagtacacatcaggaagacaggagaagaagctagcatgaagaccatcattgctttgagctacattttctgtctggctctcggccaagaccttccaggaaatgacaacagcacagcaacgctgtgcctgggacatcatgcggtgccaaacggaacactagtgaaaacaatcacagatgatcagattgaagtgactaatgctactgagctagttcagagctcctcaacggggaaaatatgcaacaatcctcatcgaatccttgatggaatagactgcacactgatagatgctctattgggggaccctcattgtgatgtttttcaaaatgagacatgggaccttttcgttgaacgcagcaaagctttcagcaactgttacccttatgatgtgccagattatgcctcccttaggtcactagttgcctcgtcaggcactctggagtttatcactgagggtttcacttggactggggtcactcagaatgggggaagcaatgcttgcaaaaggggacctggtagcggttttttcagtagactgaactggttgaccaaatcaggaagcacatatccagtgctgaacgtgactatgccaaacaatgacaattttgacaaactatacatttggggggttcaccacccgagcacgaaccaagaacaaaccagcctgtatgttcaagcatcagggagagtcacagtctctaccaggagaagccagcaaactataatcccgaatatcgggtccagaccctgggtaaggggtctgtctagtagaataagcatctattggacaatagttaagccgggagacgtactggtaattaatagtaatgggaacctaatcgctcctcggggttatttcaaaatgcgcactgggaaaagctcaataatgaggtcagatgcacctattgatacctgtatttctgaatgcatcactccaaatggaagcattcccaatgacaagccctttcaaaacgtaaacaagatcacatatggagcatgccccaagtatgttaagcaaaacaccctgaagttggcaacagggatgcggaatgtaccagagaaacaaactagaggcctattcggcgcaatagcaggtttcatagaaaatggttgggagggaatgatagacggttggtacggtttcaggcatcaaaattctgagggcacaggacaagcagcagatcttaaaagcactcaagcagccatcgaccaaatcaatgggaaattgaacagggtaatcgagaagacgaacgagaaattccatcaaatcgaaaaggaattctcagaagtagaagggagaattcaggacctcgagaaatacgttgaagacactaaaatagatctctggtcttacaatgcggagcttcttgtcgctctggagaatcaacatacaattgacctgactgactcggaaatgaacaagctgtttgaaaaaacagggaggcaactgagggaaaatgctgaagacatgggcaatggttgcttcaaaatataccacaaatgtgacaacgcttgcatagagtcaatcagaaatgggacttatgaccatgatgtatacagagacgaagcattaaacaaccggtttcagatcaaaggtgttgaactgaagtctggatacaaagactggatcctgtggatttcctttgccatatcatgctttttgctttgtgttgttttgctggggttcatcatgtgggcctgccagagaggcaacattaggtgcaacatttgcatttgactcgagaaaggagagaaggctaatgtgctaattgggcaaggagacgtggtgttggtaatgaaacggaaacgggactctagcatacttactgacagccagacagcgaccaaaagaattcggatggccatcaattagtgtcgaatagtttaaaaacgaccttgtttctact

SEQ ID NO: 127 - DNA, 1248 bp, Artificial Sequence
  Chimeric influenza virus gene
agcgaaagcaggcaaaccatttgattggttgtcaatccgaccttacttttcttaaaagtgccagcacaaattgctataagcacaactttcccttatactggagaccctccttacagccttgggacaggaacaggatacaccttggttgctagcatgacttcgaaagtttatgatccagaacaaaggaaacggatgataactggtccgcagtggtgggccagatgtaaacaaatgaatgttcttgattcatttattaattattatgattcagaaaaacatgcagaaaatgctgttatttttttacatggtaacgcggcctcttcttatttatggcgacatgttgtgccacatattgagccagtagcgcggtgtattataccagaccttattggtatgggcaaatcaggcaaatctggtaatggttcttataggttacttgatcattacaaatatcttactgcatggtttgaacttcttaatttaccaaagaagatcatttttgtcggccatgattggggtgcttgtttggcatttcattatagctatgagcatcaagataagatcaaagcaatagttcacgctgaaagtgtagtagatgtgattgaatcatgggatgaatggcctgatattgaagaagatattgcgttgatcaaatctgaagaaggagaaaaaatggttttggagaataacttcttcgtggaaaccatgttgccatcaaaaatcatgagaaagttagaaccagaagaatttgcagcatatcttgaaccattcaaagagaaaggtgaagttcgtcgtccaacattatcatggcctcgtgaaatcccgttagtaaaaggtggtaaacctgacgttgtacaaattgttaggaattataatgcttatctacgtgcaagtgatgatttaccaaaaatgtttattgaatcggacccaggattcttttccaatgctattgttgaaggtgccaagaagtttcctaatactgaatttgtcaaagtaaaaggtcttcatttttcgcaagaagatgcacctgatgaaatgggaaaatatatcaaatcgttcgttgagcgagttctcaaaaatgaacaataactcgagcccgaattgatgcacggattgatttcgaatctggaaggataaagaaagaagagttcactgagatcatgaagatctgttccaccattgaagagctcagacggcaaaaatagtgaatttagcttgtccttcatgaaaaaatgccttgtttctact

SEQ ID NO: 128 - DNA, 89 bp, Artificial Sequence
  Primer
cagctagcatggacgttaacccaactctgttatttctgaaggtaccggcgcagaacgccatcagtacgacctttccttatactggagac

SEQ ID NO: 129 - DNA, 66 bp, Artificial Sequence
  Primer
gtctcgagctacttctgtctccgaagttcctcgattgtactgcaaattttcatgatctcagtgaac

SEQ ID NO: 130 - DNA, 55 bp, Artificial Sequence
  Primer
cagctagcatggagcggatcaaggagttgcggaacttgatgtcgcagtctcgcac

SEQ ID NO: 131 - DNA, 65 bp, Artificial Sequence
  Primer
tgtgaatccgtcaagatagagctatctctctttctcttcatcactagtaccacgtctccttgccc

SEQ ID NO: 132 - DNA, 60 bp, Artificial Sequence
  Primer
gactcgagctagttaatagccatacggatcctcttagttgccgtttgtgaatccgtcaag

SEQ ID NO: 133 - DNA, 87 bp, Artificial Sequence
  Primer
cagctagcatggaggacttcgtaaggcagtgttttaacccaatgatcgttgaactcgcagagaagacgatgaaggagtatggggagg

SEQ ID NO: 134 - DNA, 66 bp, Artificial Sequence
  Primer
gtctcgagctatgatagcgcgtgcgtcaaaaaagaattaaaccagctggcgttaagcaaaacccag

SEQ ID NO: 135 - DNA, 41 bp, Artificial Sequence
  Primer
cagctagcatgaagaccatcattgctttgagctacattttc

SEQ ID NO: 136 - DNA, 42 bp, Artificial Sequence
  Primer
gtctcgagtcaaatgcaaatgttgcacctaatgttgcctctc